European Patent Specification EP 4 003 427 B1, published September 17, 2025. Title: SAPONIN DERIVATIVES WITH IMPROVED THERAPEUTIC WINDOW. Applicant: Sapreme Technologies B.V. Charité - Universitätsmedizin Berlin. The sequence listing filed with the application follows.

SEQUENCE LISTING (5 sequences)

SEQ ID NO: 1 - protein, 18 aa, Artificial Sequence
  Customized peptide
SESDDAMFCDAMDESDSK

SEQ ID NO: 2 - DNA, 16 bp, Artificial Sequence
  HSP27 BNA oligo
ggcacagccagtggcg

SEQ ID NO: 3 - DNA, 16 bp, Artificial Sequence
  HSP27 LNA oligo
ggcacagccagtggcg

SEQ ID NO: 4 - DNA, 20 bp, Artificial Sequence
  HSP27 Primer Forward
gcagtccaacgagatcacca

SEQ ID NO: 5 - DNA, 20 bp, Artificial Sequence
  HSP27 Primer Reverse
taaggctttacttggcggca